European Patent Specification EP 4 441 237 B1, published March 26, 2025. Title: Verfahren zur Herstellung von Taurin. Applicant: Wacker Chemie AG. The sequence listing filed with the application follows.

SEQUENCE LISTING (2 sequences)

SEQ ID NO: 1 - DNA, 1566 bp, Cyprinus carpio
  CDS (31)..(1530)
gttaacaatttcacacaggaaacagaattcatgagttcgtccaaggaatatatgaatggccacgtgcatctggaggagagtgatatgtatgaatccgatggcaaactgtttctgacggaagcctttaacgttatcatggaagaaattttgcacaaaggtaccgattcggaagagaaagtgtgtgagtggaaagatcccgatcagctgcgtgccctcttggatctggatctgcgtgaacatggggaatcacataaacagctgcttcaacgcgtgcgtgacgttgcacgctattctgtcaaaacctgtcatccgcgcttcttcaatcagctgtttgccggcgtagactatcacgctcttaccggacgcttgctgaccgaaaccctgaatacgagtcagtacacttacgaagtcgctccggtgtttgttcttatggaagaggaagtgctttgcaaattacgcagcctcgtcggatggtctgaaggcgacggtattttctgtcctggcggcagcatgtccaacatgtatgcgatgaatgtggctcgttattgggctttccctcaggttaaaacgcagggtttatgggcaacgccacgtatggcgattttcacctctcaacagggccattacagcatgaagaaagcggcagcctttctgggtattggcacagacaatgtgttcatcgtacaggtcgatgaaagcgggagtatgcgtcctgaggatctcgaagcgaaaatcgtacaagcgaaaagccaggatgccgttcccttctttgtgaacgcaacagccggtacaaccgttcaaggtgcctttgatccgctgaatcgtattgcggacatctcagaacgcaacggcatgtggatgcacgtcgatgcggcttggggtggttcagtgctgtttagcaagaagcacaaacatctggttgcgggcattgaacgtgcaaacagcgtgacttggaatccgcacaaaatgctgctggccgggttacagtgttctgtcgtactgtttcgcgataccacgaatttactgatgcactgccattcggccaaagcgacgtacctcttccaacaagacaagttttacgacacttcgcttgatactggggacaaaagcattcagtgcggtcgcaaggtggattgcttgaaactgtggctgatgtggaaagcgattggcacccatgggttatccgagcgtgtagagaaagcgtttgctttagcacgctatctggtcgaagaaatggaaaagcgcgacaacttcaagctggtgtgcaaaggtccgtttgtaaacgtgtgcttttggtttatcccgccgtcactccgccgcaaagaaaactccgcggattaccaagaacggttgtcgaaagtggcaccggttatcaaagagcggatgatgaaacgtggaacgatgatggtgggttatcagccaatggatggccatgtcaacttctttcgcatggttgttgtcagtccacagttgaccaccaaagacatggacttcttcctggatgagattgaagatctgggcaaagacctgtaagcttggctgttttggcggatgagagaagatatc

SEQ ID NO: 2 - protein, 500 aa, Cyprinus carpio
MSSSKEYMNGHVHLEESDMYESDGKLFLTEAFNVIMEEILHKGTDSEEKVCEWKDPDQLRALLDLDLREHGESHKQLLQRVRDVARYSVKTCHPRFFNQLFAGVDYHALTGRLLTETLNTSQYTYEVAPVFVLMEEEVLCKLRSLVGWSEGDGIFCPGGSMSNMYAMNVARYWAFPQVKTQGLWATPRMAIFTSQQGHYSMKKAAAFLGIGTDNVFIVQVDESGSMRPEDLEAKIVQAKSQDAVPFFVNATAGTTVQGAFDPLNRIADISERNGMWMHVDAAWGGSVLFSKKHKHLVAGIERANSVTWNPHKMLLAGLQCSVVLFRDTTNLLMHCHSAKATYLFQQDKFYDTSLDTGDKSIQCGRKVDCLKLWLMWKAIGTHGLSERVEKAFALARYLVEEMEKRDNFKLVCKGPFVNVCFWFIPPSLRRKENSADYQERLSKVAPVIKERMMKRGTMMVGYQPMDGHVNFFRMVVVSPQLTTKDMDFFLDEIEDLGKDL